European Patent Application EP 4 130 023 A1, published February 8, 2023. Title: L-Glutamate oxidase mutant. Applicant: Ajinomoto Co., Inc. The sequence listing filed with the application follows.

SEQUENCE LISTING (5 sequences)

SEQ ID NO: 1 - protein, 687 aa, Streptomyces sp. X-199-6
ANEMTYEQLARELLLVGPAPTNEDLKLRYLDVLIDNGLNPPGPPKRILIVGAGIAGLVAGDLLTRAGHDVTILEANANRVGGRIKTFHAKKGEPSPFADPAQYAEAGAMRLPSFHPLTLALIDKLGLKRRLFFNVDIDPQTGNQDAPVPPVFYKSFKDGKTWTNGAPSPEFKEPDKRNHTWIRTNREQVRRAQYATDPSSINEGFHLTGCETRLTVSDMVNQALEPVRDYYSVKQDDGTRVNKPFKEWLAGWADVVRDFDGYSMGRFLREYAEFSDEAVEAIGTIENMTSRLHLAFFHSFLGRSDIDPRATYWEIEGGSRMLPETLAKDLRDQIVMGQRMVRLEYYDPGRDGHHGELTGPGGPAVAIQTVPEGEPYAATQTWTGDLAIVTIPFSSLRFVKVTPPFSYKKRRAVIETHYDQATKVLLEFSRRWWEFTEADWKRELDAIAPGLYDYYQQWGEDDAEAALALPQSVRNLPTGLLGAHPSVDESRIGEEQVEYYRNSELRGGVRPATNAYGGGSTTDNPNRFMYYPSHPVPGTQGGVVLAAYSWSDDAARWDSFDDAERYGYALENLQSVHGRRIEVFYTGAGQTQSWLRDPYACGEAAVYTPHQMTAFHLDVVRPEGPVYFAGEHVSLKHAWIEGAVETAVRAAIAVNEAPVGDTGVTAAAGRRGAAAATEPMREEALTS

SEQ ID NO: 2 - DNA, 2064 bp, Streptomyces sp. X-119-6
gccaacgaaatgacctacgaacagcttgcacgcgaactgttactggtgggaccggcccctaccaacgaggacctcaaactgcgttatctggatgtgctgattgacaatggtctgaacccgccgggcccacccaaacgcattctgatcgtgggtgcaggcatcgcgggtctggtggctggggacttgctgacccgtgcaggccatgatgtaaccatccttgaggcgaacgcgaatcgcgtgggtgggcggatcaaaacctttcatgcgaagaaaggtgaacccagcccgttcgcggacccagcccagtatgccgaagcaggcgctatgcggctgccgtcgtttcacccacttacgctcgccctgatcgataaattgggcttaaaacgtcgcctgttcttcaatgtcgatattgacccgcagaccggaaaccaggatgcgccggttccgccggtcttttataaatcgtttaaagacggtaagacgtggaccaacggtgccccaagccccgaatttaaagagcccgataaacgcaatcatacctggattcgcaccaaccgcgaacaggtacgtcgcgcccaatacgcgactgatccaagtagtattaacgaaggctttcacctgactggctgcgagactcgcttaaccgtatcagacatggtgaatcaagccctggaaccggtgcgcgattattactctgtcaaacaggatgatggcacccgtgtcaacaaaccttttaaggaatggctggccggttgggcggacgtggtccgtgatttcgatggctactctatgggccgcttcttgcgcgagtacgcagaatttagcgatgaagcagtcgaagcaattggcacgatcgagaatatgacgagtcgcttacatctggccttctttcactcgttcctcgggcgtagcgatatcgacccgcgtgctacatactgggaaatcgagggcggttcacgcatgctgcccgaaactctggctaaggatctgcgtgatcagattgtgatgggtcagcgtatggtacgcttagagtattatgatccaggacgtgacggccatcatggtgaactgactggcccaggtggcccagcggtggccattcaaaccgttccggagggcgaaccgtatgcggcgacccaaacatggaccggggatctcgcgattgtgaccattccgttttcctcactgcgctttgttaaagttacaccgccgttctcctacaagaaacgccgtgcagtaattgaaacgcattacgatcaagccaccaaagttctccttgaattctctcgccgttggtgggaatttaccgaagcggattggaaacgcgaattggacgcgatcgcacctggtctgtacgactactatcagcaatggggcgaagatgatgccgaggccgcgctcgccttaccgcagtcggttcgtaatctgcctacaggtttgctgggcgcacaccctagtgttgatgagtcacgcattggagaggaacaggtagaatactaccgtaattccgaacttcgcggcggagttcgcccggctacgaatgcctatggtggaggttctaccacggacaatccgaaccggtttatgtattatccgagccacccagtgcctggtacgcaaggcggggtagtgttggctgcttattcgtggagtgatgatgcggcgcgttgggacagctttgacgacgctgagcgctatgggtatgcgctggaaaacttacaatccgtccatggccgccgcatcgaggttttctacacaggagcaggccagacacagagctggttgcgtgatccgtatgcttgtggggaggcagctgtttatacgcctcatcagatgacggcattccacctggatgtggttcgccccgaaggcccggtgtattttgctggggaacacgttagcctgaaacatgcatggattgagggcgcggtggaaaccgcggtccgggcggcgattgcggtcaacgaagcgccggtgggtgatacgggtgtcactgccgcagctggtcgtcgtggggccgccgcggccactgaaccgatgcgggaagaagcgctgacgtcctaa

SEQ ID NO: 3 - protein, 629 aa, Artificial Sequence
  Truncated L-glutamate oxidase mutant
ANEMTYEQLARELLLVGPAPTNEDLKLRYLDVLIDNGLNPPGPPKRILIVGAGIAGLVAGDLLTRAGHDVTILEANANRVGGRIKTFHAKKGEPSPFADPAQYAEAGAMRLPSFHPLTLALIDKLGLKRRLFFNVDIDPQTGNQDAPVPPVFYKSFKDGKTWTNGAPSPEFKEPDKRNHTWIRTNREQVRRAQYATDPSSINEGFHLTGCETRLTVSDMVNQALEPVRDYYSVKQDDGTRVNKPFKEWLAGWADVVRDFDGYSMGRFLREYAEFSDEAVEAIGTIENMTSRLHLAFFHSFLGRSDIDPRATYWEIEGGSRMLPETLAKDLRDQIVMGQRMVRLEYYDPGRDGHHGELTGPGGPAVAIQTVPEGEPYAATQTWTGDLAIVTIPFSSLRFVKVTPPFSYKKRRAVIETHYDQATKVLLEFSRRWWEFTEADWKRELDAIAPGLYDYYQQWGEDDAEAAGGVRPATNAYGGGSTTDNPNRFMYYPSHPVPGTQGGVVLAAYSWSDDAARWDSFDDAERYGYALENLQSVHGRRIEVFYTGAGQTQSWLRDPYACGEAAVYTPHQMTAFHLDVVRPEGPVYFAGEHVSLKHAWIEGAVETAVRAAIAVNEAPVGDTGVTAAAG

SEQ ID NO: 4 - protein, 5 aa, Artificial Sequence
  Peptide linker
GGGGS

SEQ ID NO: 5 - protein, 10 aa, Artificial Sequence
  Peptide linker
GGGGSGGGGS